European Patent Application EP 4 316 511 A1, published February 7, 2024. Title: Nasal vaccine coated with nanogels. Applicant: The University of Tokyo HanaVax Inc. The sequence listing filed with the application follows.

SEQUENCE LISTING (6 sequences)

SEQ ID NO: 1 - protein, 540 aa, Human norovirus
MKMASSDANPSDGSAANLVPEVNNEVMALEPVVGAAIAAPVAGQQNVIDPWIRNNFVQAPGGEFTVSPRNAPGEILWSAPLGPDLNPYLSHLARMYNGYAGGFEVQVILAGNAFTAGKVIFAAVPPNFPTEGLSPSQVTMFPHIVVDVRQLEPVLIPLPDVRNNFYHYNQSNDPTIKLIAMLYTPLRANNAGDDVFTVSCRVLTRPSPDFDFIFLVPPTVESRTKPFSVPVLTVDEMTNSRFPIPLEKLFTGPSSAFVVQPQNGRCTTDGVLLGTTQLSPVNICTFRGDVTHITGSHNYTMNLASQNWSNYDPTEEIPAPLGTPDFVGKIQGMLTQTTRTDGSTRGHKATVYTGSADFAPKLGRVQFETDTNNDFEANQNTKFTPVGVIQDGGTTHRNEPQQWVLPSYSGRNTPNVHLAPAVAPTFPGEQLLFFRSTMPGCSGYPNMDLDCLLPQEWVQYFYQEAAPAQSDVALLRFVNPDTGRVLFECKLHKSGYVTVAHTGQHDLVIPPNGYFRFDSWVNQFYTLAPMGNGAGRRRAL

SEQ ID NO: 2 - DNA, 1623 bp, Human norovirus
atgaagatggcgtcgagtgacgccaacccatctgatgggtccgcagccaacctcgtcccagaggtcaacaatgaggttatggctctggagcccgttgttggtgccgccattgcggcacctgtagcgggccaacaaaatgtaattgacccctggattagaaacaattttgtacaagcccctggtggagagtttacagtatcccctagaaacgctccaggtgaaatactatggagcgcgcccttgggccctgatctaaatccctacttatctcacttggccagaatgtacaatggttatgcaggtggttttgaagtgcaggtaattctcgcggggaacgcgttcaccgccgggaaggtcatatttgcagcagtcccaccaaattttccaactgaaggcttgagccccagccaggtcactatgttcccccatatagtagtagatgttaggcaactagaacctgtgttgattcccttacccgatgttaggaataatttctatcattacaatcaatcaaatgaccccaccattaagttgatagcaatgttgtatacaccacttagggctaataatgctggggatgatgtcttcacagtttcttgccgagttctcacgagaccatcccccgattttgatttcatatttctagtgccacccacagttgagtcaagaactaaaccattctctgtcccagttttaactgttgatgagatgaccaattcaagattccccattcctttggaaaagttgttcacgggtcccagcagtgcctttgttgtccaaccacaaaacggtaggtgcacgactgatggcgtgctcctaggcaccacccaactgtctcctgtcaacatctgcaccttcagaggagatgtcacccatatcacaggtagtcataactacacaatgaatttggcttctcaaaattggagcaattacgacccaacagaagaaatcccagcccctctagggactccagactttgtggggaagattcaaggcatgcttacccaaaccacaaggacagatggttcaacacgcggccacaaagccacagtgtacactgggagcgccgactttgctccaaaactgggtagagttcaatttgaaactgacacaaacaatgattttgaagctaaccaaaacacaaagttcaccccagttggtgtcatccaagatggtggcaccacccaccgaaatgaaccccaacagtgggtgctcccaagttactcaggcaggaacactcctaatgtgcatctggcccccgctgtggcccccacttttccgggtgagcaactcctcttcttcagatccaccatgcccggatgcagcgggtaccccaacatggatttggattgtctgctcccccaggaatgggtgcagtacttctaccaagaggcagccccagcacaatctgatgtggctctgctaagatttgtgaatccagacacaggtagggttttgtttgaatgtaagcttcataaatcaggctatgttacagtggctcacactggccaacatgatttggttatcccccccaatggttattttaggtttgattcctgggtcaaccagttttacacgcttgcccccatgggaaatggagcggggcgtagacgtgcactgtaa

SEQ ID NO: 3 - protein, 540 aa, Human norovirus
MKMASNDAAPSNDGAAGLVPEGNNETLPLEPVAGAAIAAPVTGQNNIIDPWIRTNFVQAPNGEFTVSPRNSPGEILLNLELGPDLNPYLAHLSRMYNGYAGGVEVQVLLAGNAFTAGKILFAAVPPNFPVEFLSPAQITMLPHLIVDVRTLEPIMIPLPDVRNTFFHYSNQPNSRMRLVAMLYTPLRSNGSGDDVFTVSCRVLTRPTPDFEFTYLVPPSVESKTKPFSLPILTLSELTNSRFPVPIDSLFTAQNNVLQVQCQNGRCTLDGELQGTTQLLPTGICAFRGRVTAQINQRDRWHMQLQNLNGTTYDPTDDVPAPLGTPDFKGVVFGMVSQRNVGNDAPGSTRAQQAWVSTYSPQFVPKLGSVNLRISDNDDFQFQPTKFTPVGVNDDDDGHPFRQWELPNYSGELTLNMNLAPPVAPNFPGEQLLFFRSFVPCSGGYNQGIIDCLIPQEWIQHFYQESAPSQSDVALIRYVNPDTGRTLFEAKLHRSGYITVAHSGDYPLVVPANGHFRFDSWVNQFYSLAPMGTGNGRRRAQ

SEQ ID NO: 4 - DNA, 1623 bp, Human norovirus
atgaagatggcgtcgaatgacgccgctccatctaatgatggtgctgctggtctcgtaccagagggcaacaacgagacccttcccctagaaccagttgcgggcgcagctatagccgcacccgtcactggccaaaataacataattgacccctggattagaacaaattttgtgcaagcaccaaatggagagttcacagtgtcacccagaaactctcctggagaaattttattaaatttagagttgggccctgatttgaacccttatttggctcatttgtcaaggatgtacaatgggtatgctggtggagtggaagttcaggttctcctggcagggaacgcgttcactgccggaaagatcctcttcgccgccgtcccgccaaatttcccagtggaattcttaagcccagcccagatcacaatgctcccacatttaatagtagatgttaggactcttgaaccaattatgatcccactccctgatgttaggaatacattcttccattatagtaaccagcctaacagccgcatgagattagtggctatgctctataccccactcagatctaatggctcaggtgatgatgtctttactgtctcttgcagggtcttgactaggcctactcctgattttgagttcacttatttagtgccaccttctgttgaatctaaaactaagcctttttccttacctattttaaccctttctgagctcacaaattcgaggtttccagtccccatcgattcgcttttcaccgcccagaataatgtgttgcaggtgcagtgtcaaaatggcaggtgtacacttgatggtgagttacaaggcacaacccagttgctcccaactggcatctgtgcattcagaggacgggtgacagcacaaattaaccaacgtgacaggtggcacatgcaactgcaaaacctcaatggtacaacatatgacccaactgatgatgtgccagccccgctgggtacacctgacttcaagggcgtcgtgtttgggatggtaagccaaagaaatgtgggtaatgatgcgcctggctcaaccagagcccaacaggcgtgggtttcaacctatagcccccaatttgtccccaaattaggttctgtcaatcttaggattagtgataatgatgatttccaattccagccgacaaaattcacaccagtgggcgtcaatgatgacgatgatggccacccgttcagacaatgggaactaccaaactattcaggggagcttaccttgaatatgaatcttgcccccccagttgctccaaattttcctggtgaacaattgttattcttcagatctttcgtgccatgctcaggaggttacaaccaaggtattatagattgtcttattccccaagaatggatccaacacttctatcaggaatcagcaccctcccagtcagacgtggccctaatcaggtatgtcaaccccgatacgggacgtacactgtttgaagcaaaattgcacagatctggttacatcactgtggctcactctggagactatcctcttgttgttccggctaatggacactttagatttgattcttgggtaaatcagttttactcactcgccccaatgggaactgggaatgggcgaaggagggctcagtaa

SEQ ID NO: 5 - protein, 542 aa, Homo sapiens
MKMASNDAAPSTDGAAGLVPESNNEVMALEPVAGAALAAPVTGQTNIIDPWIRANFVQAPNGEFTVSPRNAPGEVLLNLELGPELNPYLAHLARMYNGYAGGMEVQVMLAGNAFTAGKLVFAAVPPHFPIENLSPQQITMFPHVIIDVRTLEPVLLPLPDVRNNFFHYNQKDDPKMRIVAMLYTPLRSNGSGDDVFTVSCRVLTRPSPDFDFTYLVPPTVESKTKPFTLPILTLGELSNSRFPVSIDQMYTSPNEIISVQCQNGRCTLDGELQGTTQLQVSGICAFKGEVTAHLHDNDHLYNVTITNLNGSPFDPSEDIPAPLGVPDFQGRVFGIISQRDKHNSPGHNEPANRGHDAVVPTYTAQYTPKLGQIQIGTWQTDDLTVNQPVKFTPVGLNDTEHFNQWVVPRYAGALNLNTNLAPSVAPVFPGERLLFFRSYIPLKGGYGNPAIDCLLPQEWVQHFYQEAAPSMSEVALVRYINPDTGRALFEAKLHRAGFMTVSSNTSAPVVVPANGYFRFDSWVNQFYSLAPMGTGNGRRRVQ

SEQ ID NO: 6 - DNA, 1629 bp, Homo sapiens
atgaagatggcgtcgaatgacgccgctccatctactgatggtgcagccggcctcgtgccagaaagtaacaatgaggtcatggctcttgaacccgtggctggtgccgccttggcagccccggtcaccggtcaaacaaatattatagacccttggattagagcaaattttgtccaggcccccaatggtgaatttacagtctctccccgaaatgcccctggtgaagtgctactgaatctagagttgggtccagaattaaatccttatctggcacatttagcaagaatgtacaatgggtatgccggtgggatggaggtgcaggtcatgttggctgggaacgcgttcacagccggcaagttggtcttcgccgccgtgccaccccacttcccgattgaaaaccttagcccacagcaaatcaccatgttccctcatgtgattatagatgtgagaaccttggaacctgttttattaccactccctgatgttaggaataacttcttccattataaccagaaagatgatcccaagatgagaattgtggctatgctttatacccccctcaggtctaatggttcaggtgatgatgtgtttacagtctcctgtagagtgttgactagaccttcccctgactttgacttcacatacctggtgccaccaacagtggagtctaaaacaaagccattcaccctcccaatcctcacacttggggaactttccaattctaggttcccagtgtctatagaccagatgtacaccagccctaatgaaattatatcagtgcagtgtcaaaatggtaggtgcacactggacggggagctccaagggacaacacaactccaagtcagtggcatttgtgctttcaaaggtgaagtgaccgcccacttacatgacaatgatcacctatataatgtcaccatcacaaacttgaatgggtccccttttgatccctccgaggatatccctgcccctctgggtgtgcctgacttccagggaagggtttttggtatcatctcccaaagagataaacacaatagtcctgggcataatgaaccagcaaacaggggacacgacgctgtggtccctacttacacagcacagtacactccaaaacttggacaaattcaaattggcacatggcaaactgacgaccttacagtcaaccaaccagtcaaattcaccccagttggactcaatgacactgaacactttaaccaatgggtggtccctaggtatgctggtgccctaaacctcaatacaaaccttgccccttctgttgctccagtatttccgggagagcgcctgctcttcttcagatcatacattcccctcaagggcggttatggaaacccagccattgattgcctactgccacaagagtgggtgcaacacttctatcaggaagcagccccttcaatgagtgaggtggccctcgtcagatacatcaacccggacactggtcgggcactgtttgaggccaagctccacagagctggtttcatgacagtctcgagcaacaccagtgccccggtggttgtgcctgccaacgggtacttcagatttgattcttgggtgaaccaattttattctctcgcccccatgggaactgggaatgggcgtagaagggtccaataa